European Patent Application EP 4 450 514 A2, published October 23, 2024. Title: COMPOSITIONS COMPRISING NOVEL PROKARYOTIC SODIUM CHANNELS AND ASSOCIATED METHODS. Applicant: DUKE UNIVERSITY. Application EP. The sequence listing filed with the application follows.

SEQUENCE LISTING (80 sequences)

SEQ ID NO: 1 - protein, 280 aa, Pseudomonas xanthomarina
MQATPVETSTRRRLQQLIEQPAVQRSILLLIVINAAILGMQTSPALVASWGELLRVLDMLILGVFVVEIAARIYVHRAAFFRDPWSLFDFTVVAIALVPASGPFSVLRALRVLRVMRMVTMVPSMRRVVGALLSAIPGLGSIAMVLALVFYVSAVIATGLFGADFPEWFGNLGRSIYTLFQVMTLESWSMGIVRPLMDVFPYAWVFFIPFILIATFTMLNLFIAIIVNAMQTVTDAEHEATQASIEAAREHIEADLHEEVRALRGEIAELKDLLRGQARR

SEQ ID NO: 2 - protein, 279 aa, Sedimenticola sp.
MAGTPPLRQRLHAFLKQPYVERTIIALILINAVILGLETSPATMSTVGHLLVAVDQAILAIFVVEIALRIYVHRLDFWRDPWSIFDFTVVAIALVPAAGPFAVLRALRVLRVLRLLTMVPSMRKVVGALLAAIPGLGSIALVLLILYYVFAVIATNLFASDYPEWFGSIGLSLYTLFQIMTLESWSMGIVRPVMEQFPFAWAFFIPFILVATFTMLNLFIAIIVNAMQSYSESEHQETVQAIQITQEHIEADLHSEVRGLRAEIRELKGLLMGQTSKGG

SEQ ID NO: 3 - protein, 283 aa, Thiohalobacter thiocyanaticus
MVEVILRDLDPASLRARAGRWIESPRVQHAIVFLIVINAIILGLETSPAVMERVGPALRLADSLILGVFVVEIAIKLFAYRLRFFTIAWNVFDFIVVGIALIPASGPLAVLRALRVLRVLRLISMVPKLRFIVEALLHAVPGIASIAGLMLLLFYVFAVMATGLFGQQFPDWFGSIGASMYTLFQIMTLESWSMGIVRPVMELYPHAWLFFVPFILIATFTMLNLFIGIIVDTMQTMHEAEHSRDRSLIEQRIEAEGGAIEDEIRGLRAEIRELKAALDRGRP

SEQ ID NO: 4 - protein, 266 aa, Labrenzia sp. VG12
MRNQVKALVTSRTWEFCIIGIIVLNAVTLGLETSHAVMNSIGPALVLIDQIILGIFVIELALRLFAHGAKFFRDPWSLFDFAIVAIALLPSNGPLAVLRSLRILRVLRLISVVPSLRRVIGGLIAALPGMGSIVVLMALVFYVFGVMATKLFGASFPEWFGDLGASLYTLFQTLESWSMIMGIVRPVMEQYPYSWLFFVPFILCTAFTVLNLFIGIIVSAMQEEHEAEADANRQAIHDETGLILEEVKAMRAELSQLRAEVERTRA

SEQ ID NO: 5 - protein, 287 aa, Thiorhodospira sibirica ATCC 700588
MAEHEGLRKRMGVWIESAAIQRLIIILILVNALILGLQTSVTLMTHFGSYLIWADRLILSVFVIELLIKLFALDRRFFKNPWNVFDLVVVSLALIPSTGPLSVLRVLRLLRLVSLLPKLRFVVEALLRAIPGIISIIGLLGLLYYVFAVIATGLFGQQFPDWFGTLGKSMYTLFQIMTLESWSMGIARPVLESYPYAWLFFIPFILVATFTILNLFIAIIVSTMQSMQEEQRAIEQQAISKTLHDDSAQIHADLLRTESENQQLREELRAVREDIRALRELLAKQNP

SEQ ID NO: 6 - protein, 282 aa, Xanthomonadaceae bacterium NML93-0399
MRETGVTEYTGLRGRLHAFIAHPKVQAGILALIVVNAILLGLETAPQIMAEAGGLIRLADRVILAVFVVEIAIRLFVHRGRFFRDPWSLFDFAVVAIALVPATGPFSVLRALRVLRVLRVLTIVPSMRRVVGALLGAVPGLLSIGMVLVLIYYVCAVIATNLFGPVFPDWFGNIGRSFYTLFQIMTLESWSMGISRPVMEEFPYAWAFFIPFILVATFTMLNLFIGVIVDAMQTVSEAEHADTLDALDRTQDHIEADVHAEVRALRDEIRSLRTLLETRSER

SEQ ID NO: 7 - protein, 277 aa, Marinomonas polaris DSM 16579
MPSSTAVVTNSMRQRLKTFIENSTIQRILLALILINAVILGLETSPDVMTTAGSFLMALDKAILAVFVIELTIRLLVHRFAFFKDGWNVFDFIVVGIALVPASGPFAVLRALRVLRVLRVLTFVPSMRKIVGALIKSLNGMLSIAMVLGLVYYVAAVMVTKLFGEAFPEWFGSLGASLYTLFQVMTLESWSMGIARPVMEAFPYAWAFFIPFILIATFTMLNLFIAVIVNAVQTMHDDEHKDELDAEKATQQQLLEQMQQLQLELKALRRDINKPQE

SEQ ID NO: 8 - protein, 269 aa, Aquimonas voraii
MKALLERALAHPFTERFVLAVILINAITLGLETDARVMARFGEWLLVLDKAALVIFCIELAAKLYVRGLRFFRDPWNVFDFVVVAIALLPASGPLSVLRALRILRVLRLITIVPSLKRVVGALLGALPGMASIVMLLVLIFYVGAVMSTKLFGEAFPEWFGSVADSFYTLFQVMTLESWSMGIVRPVMEVYPYSWLFFIPFILATSFTALNLFIGVVVSAMQAEIDADRERVVEEAVAKGEEPLVEEVRALRAEIARLSQRFEGTDRPA

SEQ ID NO: 9 - protein, 264 aa, Fulvimarina pelagi HTCC2506
MQERLQHLFRSRRWEQFIIGLIVVNAIFLGLETSDAVMRNIGGLLLAFDTAILAVFVIEIVGRIYAFRGAFFRDPWSIFDFTVVGIALLPATGPLTVLRALRILRVLRLISVIPSLRRVIGGLIAALPGMGSIIALLAITFYIFAVMATKLFGDTFPQWFGDMGASIYTLFQVMTLESWSMGIVRPVMEVHPYAWLFFVPFILSTTYAVLNLFIGVIVSAMQGEHEASIDAEHEKRHNENTEILAEVKALRAELAEMRAAKAEG

SEQ ID NO: 10 - protein, 295 aa, Rheinheimera sp. SA_1
MTNSLPDAPTGLQARIINLVEQNWFGRFILTLILINAVLLGMETSASLMAQYGPLLVSLDKLLLGIFVLELLLRIFAYRSEFFKDAWSLFDFAVVAIALIPASGPLAVLRSLRVLRVLRVLSIVPSMKRVVSALLGSMPGLASIGMVLVLIYYVFAVIATKIFGTAFPEWFGTIGASFYTLFQVMTLESWSMGISRPVMEMFPYAWLFFIPFILVATFTMLNLFIAIIVNTMQTFSDEEHALERALDKQAQDQEQQQMHEELKTIRQELQQLQALLRSSPGMQPHAPSNPDQPSD

SEQ ID NO: 11 - protein, 266 aa, Neptunomonas antarctica
MHAKLKLLIENPVTQRIIISLIVINAVLLGLETSGAIMAAAGTYIVLLDKAILGVFVVEIVSRIYIYRLNFWKDPWSLFDFAVVSIAIVPSSGAFSVLRALRVLRVLRLLTMVPSMRRVVGALLSAVPGLISIAMVLLIIYYVFAVISTNLFAEQYPQWFGSLGLSLYTLFQIMTLESWSMGIARPVMETFPYAWAFFIPFILVATFTMLNLFIAIIVNAMQSFNEEERKETIDAVNVLDNDLQGELKLLRQEIRELRQFLTNKAL

SEQ ID NO: 12 - protein, 265 aa, Rhizobiales bacterium
MDRLRAFITSRRTEYFITGLIIINAITLGLETDATIAANFGDALHIFDQFILGVFVVELMLRILVHRTSFFKDPWNLFDFLIVTIALLPSSGSLSVLRALRILRVLRLITFVPTLRRVVGALIGALPGMGSIILLMALVYYVFAVMATKLFGETFPQWFGTLGESAYTLFQIMTLESWSMGIVRPVMEQFPLAWLFFVPFILSTTFTVLNLFIGIIVAAMQTEHDAEAELERQALHEENVNVLEEVKALRKEISTLHDLVKTNRA

SEQ ID NO: 13 - protein, 274 aa, Bauldia litoralis
MSAWLRSIVDDPRAERVIMVLIVINAVILGLETSETIMASHGWLLETLDRAILAVFVVEIAARIIAYRGAYFRDPWNVFDFIVVAIALVPATETFSVLRALRVLRVLRLVTRVPSLRRVVGGLITALPGMGSVVALLSLLFYVFAVMATKLFGEQFPDWFGSIGASAYSLFQIMTLESWSMGIVRPVMETYPYAWAFFVPFIVITTFAVLNLFIGIVVNAMQAEHEKAVNEERAAERDMIHDETAPLVEEIKALRVEMAALRQRIENPAVRPPE

SEQ ID NO: 14 - protein, 274 aa, Thiocapsa marina 5811
MSSREQVGAWIESTRIQRIIIVLILVNAVTLGLETSSRIMASYGGFLHLLDRVILAAFVAEILLKLFAHGLGFFRRGWNLFDFTVIAIALIPASGPLAVLRALRVLRVLRLVSVSPRLRFVVEALLKALPGIASIASLMLLLFYVAAVIATGLFGTGFPQWFGTLGRSMYTLFQIMTLESWSMGIVRPVMDVHPYAWLFFIPFILIATFTMLNLFIGIIVDTMQTLHDDQHAAERERIEQTVHSDTRAVELEVRALREEIEGLRRDLAMRAKQS

SEQ ID NO: 15 - protein, 272 aa, Solemya velesiana gill symbiont
MSSESLRYRAGVWIESKPVQNFIIALIVINAVTLGLQTSSSWMAQSGGLLLQLDNLILAVFVAEIGIKLFAFRLGFFKTGWNNFDFIVVGIALVPASGPLAVVRALRILRVLRMISMVPRLRFVVEALLHAIPGISSIGLLMLIIFYVFAVMATTLFGGDFPEWFGSIGASMYTLFQVMTLESWSMGIVRPVMELFPYAWLYFIPFILIATFTMLNLFIGIIVDTMQTMHQADHDEEREHIEQVVHEDTGELANEMRQLRAELAGMRASLGK

SEQ ID NO: 16 - protein, 283 aa, Brevundimonas sp.
MDRLRQIVTSPRTERFILALIILNAITLGLETSSWVMDRIGPVLLVLDKIVLAIFVVEVVARIAVHRLAFFKDPWSLFDFGVVAIALVPAAGPFSVLRALRILRVLRMITIVPSLKRVVGALISALPGMGSIVLLMGLIFYVASVMATKLFGADFPQWFGSIPASAYSLFQIMTLESWSMGIVRPVMEVHPYAWMFFVPFILCTTFTMLNLFIGIVVNAMQAEHEEEAKAERHKLEEDLRLASEERQKAHAEDVADMAALRGELAELRQAMTDLTTSLTRRPG

SEQ ID NO: 17 - protein, 296 aa, Betaproteobacteria bacterium HGW-Betaproteobacteria-16
MSTDTLPSHGLRQRCHAFLSQPLVQHGILALIVLNAVFMGLETSASVMAEVGPWLLAVDKVILGVFVLELAVRLYVHRSAFFRDPWSLFDFAVVAIALVPASGPFAVLRALRVLRVLRVLTIVPSMRRVVGALLSAIPGLSSIAMVLMLVFYVFAVIATHLFGQQFPDWFGHLGRSLYTLFQVMTLESWSMGISRPVMEESPYAWAFFIPFILFATFTMLNLFIAIIVNAMQTFTESEHQATVGAVETVGQSIEHELHAEVQSLRQEIGELKTMLRASSLAGAFVAPNAPTSGNSG

SEQ ID NO: 18 - protein, 275 aa, Pusillimonas sp.
MNATSLSLQQRTRKLVEHPRFTGTILTLIILTAIILGMETSPTVVAQWGPTLGLINNLFLAVFVVELVLRIYAWRTRFFVDPWSLFDLIVVGISLVPASGPLAILRALRVLRVLRLVSAVPAMRKVVAALLGALPGLGSIVVLLLLIYYVAAVIATNIFGADFPDWFGTLGRSFYTLFQIMTLESWSMGISRPVMDTFPWAWAFFIPFILIATFTMLNLFIAIIVNTMQTFHEAEQAEQQWEKDRLEQADKDYLHDQLERIQKQLDQLSRNLEKS

SEQ ID NO: 19 - protein, 283 aa, Lautropia sp. SCN 70-15
MIPSAAAGAGWRRRLADLLEAPRMQGALIALILVNAAVLGLETSPSVMARWGGLLVRIDTAILAVFVVEIALRLVARGPRFFRDPWAVFDFVVVGIALLPASGPFAVLRALRVLRVLRLMTFVPSMRRVVGGLLAAIPGLSSVFAVIALIFYVGSVMATKLFGGQFPEWFGSLGASAYTLFQVMTLESWSMGIARPVMEAFPHAWAFFVPFILIATFTMLNLFIAVIVNAIQAEHAAEHETEVRDIESAVSAHADERADALHVEIRALRAEVARLAALLEKRG

SEQ ID NO: 20 - protein, 278 aa, Ectothiorhodospira sp. BSL-9
MHAVAGPRARVGAFIESDRIQRWIIALILINAAVLGLETSPTVMEHTVGPWLLVADKIILGIFVVEILLKLFAQGWGFFRRPWNVFDFLVVGIALVPASGPMAVLRVLRLLRLVSMMPKLRFIVEALLKAIPGILSILGLLVLLFYVFAVIATGLFGKSFPEWFGNLGQSMYTLFQVMTLESWSMGIARPVMEEYNWAWVFFVPFILIATFTILNLFIAIIVNTMQSMQEDQQQFEHDTIEEVVHAENTQLHEDLKALRQEIRELRKEISSDRPSGPG

SEQ ID NO: 21 - protein, 291 aa, Alphaproteobacteria bacterium HGW-Alphaproteobacteria-11
MTTVETNSNGLRARVAALVERSLFQHFVTAVILVNAVTLGLETSASAMAAAGPLLIALDRIALSIFVVELALKLFAQRTRFFRDGWNIFDFIIVGIALVPAAGPFSVLRALRILRVLRLLSVVPSLRKVIASLIGALPGMGSIIAVLFLVFYVGAVLATKLFGASFPDWFGTIGGSMYSLFQIMTLESWSMGIVRPVMEVYPYAWIFFVPFIVMTSFMVLNLFIAIIVNSMQALHEEEHNRAQDERERLAREERAAIEKRAHAEREATLEGVRALRAELAELRALIEARPG

SEQ ID NO: 22 - protein, 285 aa, Betaproteobacteria bacterium HGW-Betaproteobacteria-11
MNTKTITDRRQRVRRWLERPLVQQTIIALIIFNALLLGLETSPAVMAHAGGLIVAIDQAILAVFVVEIALRLYAYRAAFWRDPWSIFDFFVVAIALIPATGPLAVLRALRVLRVLRLLAMVPSMRRVVGALLVAVPGPGSIALVLLIIYYVFAVIATNLFATSYPDWFGDIGRSLYTLFQIMTLESWSMGIVRPVMESFSYAWAFFIPFILIATFTMLNLFIAIIVNAMQMVSEADRCNAAQTLEHQSERIEGELHAEMGRLRVEIQALRAMLSITPAPGQTKPS

SEQ ID NO: 23 - protein, 280 aa, Methyloligella halotolerans
MQEATLPSGQNVIERLRRLVESRRFTGFITAVILFNAVTLGLETWSYAMEVAGGLLVAIDRIVLAIFVFEMIAKLLVYRQAFFRSGWNIFDLTIVGIALVPAAGPLTVLRALRILRVLRLLSVVPQMRSVVAALIGAIPGMGSIAAVMSLIFYVGSVLATKLFGAAFPDWFGSIGASAYSLFQIMTLESWSMGIVRPVMEVYPWAWLFFVPFILITTFAVLNLVVAVIVNSMQTLHEAEQKEEREAERQIVHEETAALTGEVRAMRQELSEIKALLGAKA

SEQ ID NO: 24 - protein, 272 aa, Martelella endophytica
MREKMLVLTKSREWESFILIVIIINAITLGFETSETIMQSFAGPALRLFDRAVLVIFVVEIAIRIYAHRLRFFRDPWSIFDFTIVVISLLPASGPLQVLRALRILRALRLLSMIPSLRRVIGGLIAALPGMGSIIVLMALVFYIFAVIATKLYGEAFPEWFGSLGATIYSLFQIMTLESWSMGIVRPVMEVYPNAWLFFVPFILSTAFTVLNLFIGIIVSAMQKEHEEELREEDRQAREPEMQELLHEVRALRSEVAALRQDQAPRPAPTTA

SEQ ID NO: 25 - protein, 279 aa, Alishewanella agri BL06
MTEITGTVERSLQQQVATWLQKNWVQRSLLSLILINAVILGLETAPGVMAVAGAPLMLLDKLILAVFVLEIALRIFAYRGAFFKDAWSLFDFTVVAIALVPASGPFAVLRALRVLRVLRVLTFVPSMKKIVGALVQSLNGMLSIAMVLGLVYYVSAVMATKLFGEAFPEWFGNIGRTLYTLFQIMTLESWSMGISRPVMEQFPYAWAFFVPFILIATFTMLNLFIAVIVNAVQSMHDEEHKEEIDAKQQLQHDLVSQMQQLQAELAALRAQLPPNNKVD

SEQ ID NO: 26 - protein, 277 aa, Alteromonadaceae bacterium
MNSDTIVTAVPVRQRLQQFIEHGTVQRMLLALILLNAFTLGLETSNAVMSLAGTAIHLLDKAILAIFVLEILVRLYVHRLAFFKDAWSVFDFVVVGIALLPASGPFSVLRALRVLRVLRVLTFVPSMKKIVGALMQSLNGMLSIAMVLGLVYYVASVMVTKLFGAAFPEWFGSLGASLYTLFQIMTLESWSMGIARPVMEQFPYAWLFFVPFILIATFTMLNLFIAVIVNAVQSMHDAEHKTEQDAEKATQLQLLQQMQQLKQQLSEVQQQLRDRSN

SEQ ID NO: 27 - protein, 290 aa, Thioalkalivibrio sulfidiphilus (strain HL-EbGR7)
MFHTPGVNPGLRERAGRWIESGPVQRVIIALILINAAILGLETDPDIMARIGDWLIGADRVILGVFVVEILIKLYAKGLRFFRNPWNVFDFLVVGIALIPASGPFAVLRILRLLRLVSMIPKLRFVVEALLRAIPGIASIFGLLIILFYVFAVIATGLFAKDHPEWFGSIGRSMYTLFQVMTLESWSMGIARPVMETHPYAWVFFVPFILVATFTILNLFIAIIVNTMQTLAEEQQKFEEKTITTVVHAESAQLHQDLTRVESENQQLHQDLRALREEIRALREELRRPG

SEQ ID NO: 28 - protein, 284 aa, Oleiphilus messinensis
MNAQLLGDTTGFRAKAHQFIENPFIQNGILVLIVINAITLGLETVPAAMQRFSNIIHTLDLVILSVFVLELLIRLYVYREKYFNDPWRAFDFVVVSIALVPATGQLAVLRALRVLRVLRIITIVPSMRRVVGALLSAIPGLTSIALVLGLIYYVFAVIATNLFAAEFPEWFGHLGRSFYTLFQIMTLESWSMGIARPVMETFPYAWAFFIPFILVATFTMLNLFIAIIVNAMQTFTEQEKQGTVEAVNEARDHIEEDMHTEMRALRREIAELKSMIRGQYRQDP

SEQ ID NO: 29 - protein, 282 aa, Rhodospirillaceae bacterium
MANLTDSAGNPGHRAWLREWVESAPFRYTVLVIIFINAIVLGLETEASVIAEVGDMLHLIDKIILWIFVVELILRMYAHGPRFFLDPWGVFDFIIVAIALFPASEEFSVLRALRILRALRLISGVPRMRRVVEALLRAVPGIGSVAALLLLVFYVFSVIATKLFGTAFPQWFGTIGESMYSLFQIMTLESWSMGIVRPVMEEYPEAWAFFVPFIIISSFTVLNLFIAIIVDSMQTLHADEEERTVERIETIVDEDTQLVSDEIARLRAEIRDLRSELNGRKS

SEQ ID NO: 30 - DNA, 843 bp, synthetic construct
  misc_feature 1..843: note = Synthetic construct
  source 1..843: mol_type = other DNA
atgcaagcgacccccgtagaaactagcactaggcgacgactccagcagcttatagagcaacccgccgtacaacgatctatacttttgttgatcgtaattaatgccgccatattgggcatgcagacatcccctgcgcttgttgctagttggggggaattgttgcgggtattggacatgttgatcctgggtgttttcgtcgtcgagatcgccgctagaatatacgttcatcgcgcagcgttctttcgggacccttggtctctgtttgacttcacagttgtcgctatcgccctcgttccggcttcagggccctttagtgtcctgcgggcgttgagggtactcagggtaatgagaatggtaacgatggtcccgagcatgcgccgagtcgtgggggctctgttgtccgctatccctggcttgggatctatagcgatggtattggccctggttttttatgtaagtgccgtgatcgcaaccggcctgtttggggccgacttccccgagtggtttgggaaccttggtaggtccatttatacgctgttccaagttatgactttggaatcctggagcatggggattgtgcggccgcttatggatgtttttccctacgcttgggttttctttattccatttattcttatcgccactttcacgatgttgaacctttttatagcaataattgtaaacgcaatgcaaaccgtcaccgatgctgagcatgaggcaacgcaagcgtccatagaagctgcgcgagaacatatcgaagctgatctccacgaagaggtaagggctcttagaggtgagattgcggagctcaaagacctccttcgcggccaggcacgcagatga

SEQ ID NO: 31 - DNA, 840 bp, synthetic construct
  misc_feature 1..840: note = Synthetic construct
  source 1..840: mol_type = other DNA
atggccggtacgcctccactgagacagaggcttcatgccttcttgaaacaaccatatgtggagcgaactattattgcgcttattctgatcaacgccgtaatactcggacttgagacatccccggctacgatgtcaaccgtcgggcatcttttggtagcggtcgaccaagcaattctcgcaatattcgtagtagaaattgcgttgagaatctatgttcacagactggatttttggcgcgacccttggagcatctttgatttcacagtcgtagcgattgcgttggttccagctgccggacccttcgcggttctcagggccttgcgcgtcctccgcgtacttcgactgttgacaatggtcccctccatgagaaaggtcgtcggggctttgttggcagcgatcccaggcttggggtctatagctcttgttctgctgatcctttattatgttttcgccgttatagccactaatttgtttgccagcgattaccccgaatggtttgggagcataggactgagtctttataccttgttccagataatgactttggaatcttggagtatgggcatcgtgagaccggtcatggaacaatttcccttcgcttgggctttcttcataccctttatacttgtggcaacttttacgatgcttaatttgttcatagcgattatcgttaacgccatgcagagctatagcgagagtgagcaccaggagactgttcaggctatccagataactcaagagcatattgaagcggacttgcactctgaagtgcgcgggcttcgcgctgaaatccgagagttgaaggggcttttgatgggtcagactagtaagggcggttga

SEQ ID NO: 32 - DNA, 852 bp, synthetic construct
  misc_feature 1..852: note = Synthetic construct
  source 1..852: mol_type = other DNA
atggtagaggttatccttcgagatttggacccagcttcccttagagcgcgagcaggcagatggatcgagtctccgagagtgcagcacgcaatcgtatttctcatcgttatcaacgcaatcattcttggactggaaacgagcccagccgttatggagcgggtagggccagcattgcgccttgcagattccctgatattgggagtatttgttgtagaaatcgcgataaaacttttcgcataccgattgagattttttacgattgcgtggaatgtattcgattttattgttgtaggaattgcgctcatcccggcttcaggacccttggccgtacttcgcgcgttgagagtgctccgggtgcttaggctcatcagcatggtcccgaagctcagattcattgttgaagcattgttgcatgcggttccgggtatagcgagtatcgcaggtttgatgctgctcctcttttatgtgtttgcggttatggctacgggactgtttggacaacagttccctgactggtttggaagtattggggcaagcatgtataccttgtttcaaataatgaccctggaatcatggagcatgggaatagttcgccccgttatggagctttacccccatgcatggttgttcttcgtcccattcattctcatcgctacatttaccatgctgaatttgttcattggcatcatagtagacacaatgcagactatgcacgaagctgagcactctcgcgacaggagcctgatcgagcaaagaatcgaggctgaaggcggcgcaatagaagatgaaatacggggactgagagcggaaatccgagaactgaaggcggctctcgacaggggacggccgtga

SEQ ID NO: 33 - DNA, 801 bp, synthetic construct
  misc_feature 1..801: note = Synthetic construct
  source 1..801: mol_type = other DNA
atgcgcaaccaagtaaaggctctcgtcactagcaggacatgggagttctgcattattgggattatcgtgctcaacgcagttacattgggactggaaacgtctcacgcggttatgaactcaatcggtcccgctcttgtgttgatagatcagattatattgggtatatttgttatcgaactggcacttcgactgttcgcacacggtgcgaaatttttccgggacccatggtcacttttcgacttcgcgattgtcgcgattgcgcttcttcccagcaatggaccgctggccgtactgcgctccttgcgcatcctgcgcgtcctgcgactcatcagcgtagttccaagccttcggcgggtcataggtggactgattgctgcgcttccagggatggggtcaatcgtggtcctcatggctttggtcttctatgtttttggcgtcatggcgacgaagttgttcggggcgtctttcccagagtggtttggagacctcggcgcttctctttacacacttttccagataatgactcttgaatcttggagcatgggcatagtccgccctgtaatggaacaatatccttattcatggcttttttttgtgccattcattttgtgtaccgctttcacggtcttgaacctgtttataggtattattgtatccgccatgcaagaagagcacgaagcagaggcggatgctaacaggcaagcaatccacgatgagacaggtctgatactcgaagaagtcaaagcgatgcgggcagagcttagccaactgagggcggaagtagagcgaactagagcgtga

SEQ ID NO: 34 - DNA, 864 bp, synthetic construct
  misc_feature 1..864: note = Synthetic construct
  source 1..864: mol_type = other DNA
atggctgagcatgagggattgcgaaagcggatgggtgtttggatcgagagtgccgcgatccaacgcctcatcatcatcttgatactggtgaacgcgcttattctcggcctccagactagcgtaaccttgatgactcacttcgggagttatctgatatgggcggaccgccttatccttagcgtattcgtaatcgagctgcttatcaagctgtttgctttggataggcgcttctttaaaaatccctggaatgtgtttgacctggtggtggtttccctcgctttgattccgagcactggacctctcagtgtccttagagttctcagattgttgcgcctggttagccttcttcctaaactgcgcttcgtagtggaagcactccttcgagctattcctggaattatctctatcattggtctgctgggtctgctctattacgtctttgctgttattgcaacaggattgttcgggcaacaattcccagattggtttggcaccctggggaagtctatgtacacattgtttcaaataatgacattggagtcatggtccatgggtatagcgcgcccggtactcgaatcttatccttacgcatggttgttttttatcccgttcatcctggtagcaacgtttaccattctcaatcttttcattgcgatcatcgtgagcactatgcagtcaatgcaagaagaacagagagcgattgaacagcaagccattagtaaaacacttcacgatgacagcgcacaaatccacgcagacctcttgcgcactgagtcagaaaaccagcagctcagggaggaacttagggcagttagagaagacatccgcgccctcagagagttgctcgccaagcagaatccgtga

SEQ ID NO: 35 - DNA, 849 bp, synthetic construct
  misc_feature 1..849: note = Synthetic construct
  source 1..849: mol_type = other DNA
atgagggagacgggtgtgacggaatacacaggtctccgagggaggctccatgcgttcattgcccaccccaaagtccaggcgggcatacttgccttgatcgtggtcaacgccattcttttgggactggaaactgctcctcagatcatggcagaagcgggcggcctcataaggttggcagatagggttatcctggccgtgttcgttgtcgaaatcgccatacgactgttcgtccacagaggcaggtttttcagggacccctggtccctttttgactttgcggtcgtcgcgatagctttggtccctgcaacgggcccatttagtgtgcttagggctcttagggtcctccgggtccttagagtattgacgatagttccatccatgcggcgcgtcgtgggtgcgcttcttggggcggtgccagggctcctctccattggaatggtcttggtgttgatttactacgtttgtgctgtaatcgctacaaatctctttgggcccgtcttccctgattggtttggcaacattgggaggtctttctacacactttttcagataatgaccctggagtcctggtcaatggggatcagtagaccagtaatggaagagtttccgtatgcgtgggcgttctttattccctttatcctggtcgccacgtttactatgctgaatctgttcataggcgtcatagttgatgcaatgcagacagtgagtgaagcggaacatgccgacacattggacgcgttggatcgaacgcaggatcacattgaagctgatgtacatgcggaagtacgggctcttagggacgaaatacggtctcttcgcacgcttttggaaacacgaagtgaacgatga

SEQ ID NO: 36 - DNA, 834 bp, synthetic construct
  misc_feature 1..834: note = Synthetic construct
  source 1..834: mol_type = other DNA
atgccatcatccactgcggtcgttactaattctatgagacagaggctcaaaacattcatcgaaaactcaacaatacaacgaatactgttggccctcatcctgataaacgccgtcatccttggtctggagacctccccagatgttatgacaaccgcagggtcttttcttatggctctggataaagcaattcttgcggtgttcgtaattgaactcacaatcaggttgttggtgcatcgattcgccttcttcaaagacggatggaatgtttttgactttatcgtggtgggcatagccctcgtccctgcaagcggcccctttgctgtcctgagagcgctccgggtattgagggttttgcgggtcctcactttcgttccttctatgagaaagatcgttggtgccttgatcaagtccctgaatggaatgctctcaattgcgatggtcctgggattggtttactatgtggcggcagtcatggttactaaactcttcggtgaggcgttcccggaatggtttgggagtctgggcgccagtctttatacactcttccaagttatgacactggagtcatggagcatgggaatcgcgcgacccgtaatggaggcgtttccttacgcatgggctttttttataccgtttattctcatcgcaactttcaccatgttgaatctgttcatcgcggtgatagtgaacgcggtgcaaactatgcatgatgacgaacacaaagatgagcttgatgctgagaaggcgacacagcaacaactgttggaacagatgcagcaacttcaactggagctgaaagcgctgcgacgggatattaacaaacctcaagaatga

SEQ ID NO: 37 - DNA, 810 bp, synthetic construct
  misc_feature 1..810: note = Synthetic construct
  source 1..810: mol_type = other DNA
atgaaggcccttctggagcgagctctggcacaccctttcacggaacggtttgttcttgctgtcattcttataaatgctattacgttggggctggagacagatgctagggtgatggctcgcttcggtgagtggcttttggtacttgataaggccgccctcgtcattttctgcattgaacttgctgccaaactctacgtgagaggactcaggttctttagggacccctggaacgtctttgacttcgtagtggtggcaatcgcacttctccccgcgtcaggccctctgtccgtgctgcgggcgttgcgcattctccgagttcttagactgataacaatcgttccatccttgaaacgggtagtaggagcccttctgggagcattgccgggcatggcaagtatagtaatgttgctcgttctgatattctatgttggggcggtaatgtccaccaaactctttggcgaagcttttccggagtggttcggtagcgtggctgactccttctataccttgttccaggtgatgactcttgaaagctggtctatgggaatagtccgcccggtaatggaggtgtatccgtatagctggctgtttttcattccattcattctggctaccagcttcacagcgttgaaccttttcattggggttgtcgtttcagctatgcaggccgagatagacgctgaccgcgaaagagtggtcgaagaggccgtggctaagggagaggagcctcttgtggaggaagtgagggctttgagagcagagatcgctaggctttctcaacgcttcgaaggcactgataggcctgcttga

SEQ ID NO: 38 - DNA, 795 bp, synthetic construct
  misc_feature 1..795: note = Synthetic construct
  source 1..795: mol_type = other DNA
atgcaggaaaggctccaacacctcttccgatcaagacggtgggaacaatttatcataggtcttatcgtcgtaaacgcaatttttctcgggctggaaaccagtgacgctgtcatgagaaatataggtggacttttgttggcgttcgatacggcaatcctggcagtatttgtaatagaaattgttggcagaatatatgcgttccggggcgctttctttagagacccttggtcaattttcgattttaccgtcgtcggtatagctctcctgcctgcaacaggacctctgactgtattgagagcattgagaatcctgcgggtactgagactcataagcgtcattccctcactccgccgggtaatcggggggctcatagcggcgctcccaggcatgggaagcatcattgccttgctggctatcacgttttacatcttcgccgtgatggccacgaaacttttcggggacacctttccgcagtggtttggggacatgggggccagcatctataccctgttccaggtcatgacactggaaagttggtcaatgggaatagtccgcccggtcatggaagtccatccctatgcttggctgttttttgtgccgtttatactttctactacttatgcagttctgaaccttttcattggggtcattgtttcagctatgcaaggagaacatgaggccagcatagacgcagaacatgaaaaaagacacaacgaaaacaccgaaattttggcggaagttaaggcgcttcgcgcggaattggccgaaatgagagcggctaaggcggagggatga

SEQ ID NO: 39 - DNA, 888 bp, synthetic construct
  misc_feature 1..888: note = Synthetic construct
  source 1..888: mol_type = other DNA
atgactaacagcttgccggacgctccaacaggcctccaggcccgaataattaatctcgttgagcaaaattggtttgggaggtttattcttacgttgatcttgattaacgctgtactgctcgggatggaaacttcagcgtctcttatggcccagtatggacctctcttggtgtccctcgataaactccttcttgggattttcgttttggagttgttgctccgaatctttgcgtatagaagtgagttctttaaggatgcctggagtctctttgactttgctgtggtagccatagccctgatcccagcctccgggcctttggctgttctgcgctcactgagagttcttagggttctcagagtcctgtccatcgtaccctcaatgaagagagtagtatcagcacttctgggcagtatgcccggtcttgcgtcaattggtatggtacttgtcctcatttactacgtatttgctgttattgcaactaaaatcttcggaacggcctttcctgaatggttcggaaccatcggggcttctttttatacgcttttccaagttatgacattggaaagttggtccatggggatttctcgccctgtcatggaaatgtttccctatgcgtggctctttttcattccgtttattttggtagccacctttacgatgctcaatctctttattgccataatagttaataccatgcagacgttctccgacgaggaacacgcccttgagagggcactcgataagcaagctcaagatcaagagcaacaacagatgcacgaagagctcaagactattcgacaagaactccaacagcttcaagcactcttgaggagttcccccggcatgcagcctcacgcaccttccaacccagaccaacccagtgattga

SEQ ID NO: 40 - DNA, 801 bp, synthetic construct
  misc_feature 1..801: note = Synthetic construct
  source 1..801: mol_type = other DNA
atgcacgctaaactcaaattgcttattgaaaatccggtgacgcaaagaataatcatcagtctgatagtaattaacgcggtactcttgggcttggaaacatcaggtgccattatggcggctgcgggcacctatattgttctgcttgacaaagcaatcttgggtgtgttcgtcgtagaaattgtatctaggatctacatatacaggctgaatttttggaaggacccgtggtcactctttgactttgccgtggtatctattgccattgttccaagttcaggggcattctctgttcttcgggcactccgcgttttgagagtgcttcgcctgctgactatggtaccctctatgaggcgggttgttggggcgcttctctcagcggtaccagggctcatcagtatagctatggtgctcctcataatttattatgtcttcgccgtaatatctaccaatctgttcgccgaacaatatccgcagtggttcggaagcctgggtctttcactgtataccctgttccagattatgactctggagtcttggagtatgggaattgcgagacccgtaatggagactttcccctacgcgtgggcgttttttattccttttatcctcgtagctacctttacgatgcttaacctctttatagcgataattgtgaatgcgatgcagtcctttaatgaggaagaaaggaaagaaacgatcgatgctgtaaatgttctcgataacgaccttcaaggagaactcaaacttctgaggcaggaaattcgcgagcttcgccagttcttgacgaataaggccctgtga

SEQ ID NO: 41 - DNA, 798 bp, synthetic construct
  misc_feature 1..798: note = Synthetic construct
  source 1..798: mol_type = other DNA
atggacaggttgcgcgcctttattacgagtcggagaaccgagtattttattaccggcctgataattataaatgctattacattgggacttgaaactgatgcaaccatagccgccaattttggggatgcgctgcatattttcgatcagttcatcctcggtgtttttgtggtcgaactgatgttgagaatcctggtgcatcggacaagcttttttaaggacccttggaatctctttgattttctcatagtcaccatagccttgcttccaagttctggaagccttagtgtcttgcgagccctgcgaatattgagggttttgaggttgatcacgtttgttcccacattgcgacgcgtggtgggtgccttgataggcgccctccctggaatgggctccattatattgcttatggccctggtctactatgtgtttgcggtgatggctactaagctttttggggaaacctttcctcagtggttcggaaccctgggcgaatcagcttatacactcttccaaattatgacgcttgaatcatggagcatgggcatagtgcggcctgttatggaacaatttcctttggcctggctgtttttcgtaccctttatcctttccacgaccttcacggtactgaacttgttcatcggtatcattgtagcagcaatgcaaaccgaacatgatgctgaggcagaactggaacgacaagcacttcacgaggagaacgtaaatgtactcgaagaagtgaaggcccttcggaaggaaatcagcacgctgcacgatctggtaaaaaccaatagagcttga

SEQ ID NO: 42 - DNA, 825 bp, synthetic construct
  misc_feature 1..825: note = Synthetic construct
  source 1..825: mol_type = other DNA
atgagcgcatggcttaggagtattgtcgatgaccccagagcggagcgagtaattatggttctgatagtgataaacgcagttattctcgggttggaaacctctgagactataatggcgtcccacggatggcttttggagacactcgaccgggctattctcgcagttttcgtagtagaaatcgcggctcgaataatcgcttaccggggggcatattttcgcgatccttggaacgtcttcgatttcatcgtggtggctatcgcactcgtacccgcaacggaaactttttcagtcttgcgcgctctgcgagttcttcgggttttgcgcctggtaactcgggttccgagcttgcggcgagtcgtaggggggttgattacggccctccccggcatgggatcagtagtagctctgttgagcttgttgttctatgtcttcgctgtgatggcaactaaactcttcggagaacaatttcctgactggttcggatcaataggagctagtgcgtattcacttttccagattatgacacttgagtcttggagtatggggattgtgaggcccgtcatggagacgtatccttacgcctgggcgttcttcgtacctttcattgtaataacgacgttcgctgtcttgaaccttttcataggtatagtcgttaatgctatgcaagctgaacatgaaaaggctgttaatgaagagcgggcagcagaacgcgacatgattcacgatgaaactgcaccgctcgtggaggaaattaaagccttgcgagttgagatggccgctcttcgccaacggatagaaaaccctgctgtacgaccgcctgaatga

SEQ ID NO: 43 - DNA, 825 bp, synthetic construct
  misc_feature 1..825: note = Synthetic construct
  source 1..825: mol_type = other DNA
atgtcatcacgcgagcaagtcggtgcttggatagaatcaacccgcatccagcgcattataattgtcctgattctcgtcaatgcggtaactcttggtctggagacgtcaagtaggatcatggcaagctacggcggcttcctccatctgttggaccgcgtcatccttgcagcattcgtcgcagagattcttttgaaacttttcgctcacggcctgggtttctttagaaggggctggaaccttttcgattttaccgtgatcgctattgctctcatcccagcgtctggacccctcgcagttctgcgagcgcttagagttttgagggttcttcgcctcgtcagtgtctcaccgagattgaggttcgtcgtggaagcgcttctcaaggcgctgcccggtattgcaagcatcgccagtctcatgttgcttcttttctatgtagcggcggtcatagcaacggggctcttcgggacgggttttccccagtggttcggaactcttggccgctcaatgtatacgttgtttcaaataatgactctggaaagctggtctatggggatcgtgagaccagtcatggacgtacacccttacgcttggttgttttttatccccttcattttgattgcaactttcaccatgttgaacctgtttatagggataattgttgataccatgcagacactgcacgatgaccagcacgcggctgaaagagagcggattgaacaaacagttcactccgatacacgcgccgttgagttggaagtgagggcccttcgcgaagagattgagggcctgcgaagagacctcgctatgagggctaagcagagttga

SEQ ID NO: 44 - DNA, 819 bp, synthetic construct
  misc_feature 1..819: note = Synthetic construct
  source 1..819: mol_type = other DNA
atgtcatcagaatctctgagatatagagcgggggtttggatagaatctaaacctgtccaaaacttcatcatagcactgatagtgataaatgcggtcacccttggtctccagacgtcttcatcatggatggcacaaagtggtggactgctccttcaactcgacaacttgattctggccgtcttcgtagcggagatcggaattaaactgttcgcctttcgattgggttttttcaaaacggggtggaataactttgatttcatagtagttggcatagctttggtgcctgcgtctggccctctcgctgtggtccgagctctgcgcatactgcgggtgcttagaatgatctctatggtcccgcgactccggttcgtagttgaagcccttctgcacgctatccccggaatcagttccatcggcttgttgatgcttatcatattctacgtctttgcggtgatggctactacccttttcggaggagattttccagagtggttcggttctataggcgcttccatgtacaccctcttccaagtaatgacactcgaaagctggagtatgggtatagtccggccggtaatggaattgtttccgtatgcctggctctatttcattccattcatactgatcgcgaccttcactatgctcaacttgttcatcggtataatagtggatacaatgcaaactatgcaccaggccgatcatgatgaagagcgcgaacatatcgaacaagttgtccatgaggacacaggggagcttgctaacgagatgaggcaactgagggcagagttggcagggatgagagcgagtctcgggaaatga

SEQ ID NO: 45 - DNA, 852 bp, synthetic construct
  misc_feature 1..852: note = Synthetic construct
  source 1..852: mol_type = other DNA
atggacagactccggcaaatagtaacgagtccccggactgagagattcatcttggcgttgataattttgaatgcgataaccctcgggctcgaaacctcatcctgggttatggatcgaattggtcccgttctccttgtgctggataaaatagtactcgcgattttcgtagtagaggtcgttgctcggattgcagtccaccgactggccttcttcaaggacccttggagtcttttcgattttggtgtcgtagcgattgccctcgtgccggctgcgggacctttcagcgtcttgagagcccttaggatacttagggtcctccgcatgataactatagtaccatcattgaagcgcgtcgtgggcgcgttgatttctgctcttcccggaatgggctccatagtacttttgatgggattgattttttatgttgccagcgttatggcgactaaactttttggcgcggacttcccacagtggtttggatctatccctgcatccgcctattctctgtttcaaatcatgaccctggagtcttggagcatgggcattgtaaggccagtgatggaagtacacccatacgcgtggatgttcttcgttccgttcatcctctgtacgacctttaccatgttgaatctgttcatcggaatcgtggtcaacgccatgcaggccgaacacgaggaagaggcgaaagccgagcgacacaaactggaagaagacctgagacttgccagcgaggaacggcaaaaggcgcacgcggaagatgttgctgacatggctgcactcagaggagagttggcggagttgcgccaggctatgacagacctgacaacgagcttgacacgccgacccggttga

SEQ ID NO: 46 - DNA, 891 bp, synthetic construct
  misc_feature 1..891: note = Synthetic construct
  source 1..891: mol_type = other DNA
atgtcaaccgacacgctgccctctcatgggctgcggcagcgatgccatgcctttctcagccaaccgttggtacaacatggaatactggcgctgatcgttcttaatgcagtctttatgggtctggagacgtctgccagtgtgatggcagaagtgggaccatggcttctcgccgtggacaaagtaatcctcggcgtttttgtattggagctcgccgttcggttgtatgtacataggagtgcctttttcagagacccgtggtcattgttcgactttgctgtcgtggccatcgcacttgtacctgcctcaggtccctttgctgtactgagggcgctccgcgtgctgagagtccttcgagtcctgaccatcgttccatcaatgaggagggtcgttggcgccttgttgagtgccattccgggtctctcatctattgccatggtactgatgctggtattctatgtctttgctgtaatcgctacacatctgtttgggcaacaattccccgattggttcgggcacctgggcaggtctctttacactctttttcaagtgatgactctcgaatcatggagcatgggaattagcagacccgtaatggaagaatcaccatacgcctgggcctttttcattccgtttatattgtttgctacctttaccatgctgaacctcttcatagccattattgtgaatgctatgcagacgtttaccgaaagtgagcaccaggcgacagtcggggccgtcgaaacggttggtcagtcaatagagcacgagctccacgccgaagttcaatctctgagacaagaaataggggagctcaaaactatgctcagagcctcatcattggcaggggcttttgtagcgcctaatgcaccgacttcaggtaattcaggatga

SEQ ID NO: 47 - DNA, 828 bp, synthetic construct
  misc_feature 1..828: note = Synthetic construct
  source 1..828: mol_type = other DNA
atgaatgcaacatctctttctctgcaacaacgaacacgaaaattggttgaacatcctcggtttacaggcacgattttgactctgatcattttgacagcgataatacttggcatggaaaccagcccaacagtcgtggcccaatggggaccgaccctcggtctgatcaacaatttgtttcttgccgtcttcgtcgtggagctcgtgcttcgaatatatgcctggaggaccagattttttgtcgacccttggagcctcttcgatttgattgtagtggggatctcacttgtaccagcctccggtccactcgctattctgagggctttgcgagtgctgcgagtattgcgccttgttagtgcggtaccggcgatgagaaaagtggttgctgctctcctcggtgctcttccaggtcttggcagtatcgtagtgcttttgcttctgatatactatgtagctgcggtcattgcgacgaatatctttggcgcagatttcccagattggttcggtacgctgggccggagtttttacacgctttttcagataatgaccttggagagctggtctatgggcataagtcgccctgtaatggatacgttcccgtgggcatgggcattttttataccctttattctgatagcgacgtttactatgctgaatctcttcatagctataatcgtgaacaccatgcaaaccttccatgaggcggagcaagcagaacagcagtgggaaaaagatcgcctggaacaggctgacaaagattatcttcatgaccagctcgaacggatacagaaacagctggaccaactgagtagaaatctcgaaaagtcttga

SEQ ID NO: 48 - DNA, 852 bp, synthetic construct
  misc_feature 1..852: note = Synthetic construct
  source 1..852: mol_type = other DNA
atgattccatccgccgcagcgggcgcaggatggaggcggaggctggccgaccttcttgaggccccgcgcatgcaaggagcactgattgcattgattttggttaatgccgcagtcttgggccttgaaacctctccctctgtgatggcccgctggggcggattgttggtgcgaattgatacggcgatattggccgtttttgtcgtagagatcgctttgagattggtcgctcgcggaccgaggttcttcagagatccttgggctgtgtttgatttcgtggtagtaggcatcgccctgttgccagcctctggtccgttcgcggtgttgagggctctccgcgttctccgagttttgagacttatgacattcgtacctagcatgcgcagggttgtcggaggattgctcgccgcaattcccggattgtcctcagtttttgcagtcattgcacttattttctacgtcggaagcgttatggcaacgaaactgtttggcggtcaatttcccgagtggttcggctctttgggcgcgtcagcgtacacgttgtttcaggttatgacgctggagagctggtcaatgggtattgcacggccagttatggaagcattccctcacgcatgggccttcttcgttccttttatccttatcgccacgttcaccatgttgaatctgtttattgccgtcatagtaaatgccatccaagcagagcacgctgcggaacatgaaacggaagttcgcgatatagagtccgctgtctctgcacatgcggatgagagggcggatgccctgcatgtcgagattcgagctttgcgggcagaggtggctagacttgcggcactgttggagaagcgggggtga

SEQ ID NO: 49 - DNA, 837 bp, synthetic construct
  misc_feature 1..837: note = Synthetic construct
  source 1..837: mol_type = other DNA
atgcacgcggtcgctggtcctagagcgagggttggcgcatttatcgagagtgaccgaatccagaggtggataattgcgttgatcctgatcaatgctgcagtcctcgggttggaaacttctccaacggtcatggagcatacggtcggtccttggttgcttgttgccgacaagatcatactcggcatctttgttgtcgagattctgttgaagcttttcgcacaggggtggggtttctttcggcgaccttggaatgtcttcgacttcctcgtggtcgggatagccctcgtccccgcgagcggtcctatggcggttttgcgagtactccgacttctgagactggtctctatgatgcccaagcttcgcttcattgtcgaggctctgttgaaggctatacccggcatcctgagtattttgggcttgttggtgctgctcttttacgtctttgcagtcattgcgacgggcctgtttggaaaatctttcccggagtggtttggtaacctgggccagtctatgtacacgctcttccaagtgatgacacttgaatcctggagtatgggcatcgcgcgacccgttatggaggaatataactgggcatgggtattcttcgttccctttatccttattgcgacatttacaatcttgaacctcttcattgcgataatagtgaacacgatgcaaagcatgcaagaggatcaacaacaatttgagcatgataccattgaggaagtggttcacgccgaaaatacacagttgcacgaagatcttaaagctttgagacaagagatacgcgaactcaggaaagaaattagctcagatagaccttcaggtcccggatga

SEQ ID NO: 50 - DNA, 876 bp, synthetic construct
  misc_feature 1..876: note = Synthetic construct
  source 1..876: mol_type = other DNA
atgacaacggtcgagacaaactctaatggtctcagggcgcgagtcgccgccttggtcgaacgctctctctttcagcacttcgttactgcggtaattctggtgaacgctgttacccttgggctcgaaacaagcgcaagtgcaatggctgctgcgggtcccctgctgattgccctggacagaatcgcgcttagtatatttgtggttgagctggctcttaaacttttcgcgcagaggacacggttcttcagggacggctggaacatctttgatttcattatcgttgggatagcgttggtgccggcggcggggccttttagtgtgctccgagctttgcgaatattgcgcgtattgcggcttctgtccgtagtaccgagtcttcgcaaggtcattgcgtctctgattggggctttgccgggaatgggtagcatcatagccgtcctttttctggtattctacgttggcgcagtactggcgacaaagctcttcggcgcttcctttccagactggttcggcactatcgggggctccatgtactctctcttccaaatcatgacactcgaaagctggtcaatgggtattgtccgaccagtaatggaggtgtatccatatgcgtggattttctttgtacctttcatcgtcatgacgtccttcatggtgcttaacttgttcatcgccattatcgtaaattctatgcaggcgctccatgaggaggagcataatagagcgcaggatgaaagagagcggctcgctcgcgaggaaagggccgcgatcgagaaaagggctcatgccgagcgagaggctacgctggaaggcgttcgggctcttagagcagaattggcggaattgcgggctcttatagaggctaggccgggatga

SEQ ID NO: 51 - DNA, 858 bp, synthetic construct
  misc_feature 1..858: note = Synthetic construct
  source 1..858: mol_type = other DNA
atgaatacgaagacaatcacagaccgccgacagagggttcgcaggtggctcgaaagacctttggttcagcagacgataattgcgctcatcatctttaacgcactgttgttgggacttgaaacctcccccgccgtgatggcgcatgctggtgggctgatagtagcaatagaccaagcaattcttgctgtgttcgttgtcgagatcgcattgaggctgtatgcctaccgggcagccttttggcgagatccatggtcaatcttcgactttttcgtggtagcgattgcgttgatcccggctactgggccgcttgcagttttgagagcacttagagtcctgcgagttttgagacttcttgcaatggtccccagcatgcggagggtcgttggagctctccttgtagccgtcccgggtcccgggagcatcgctctcgtacttcttatcatctattatgtattcgccgtaatcgcaactaacctgttcgctacttcctacccggattggtttggagatatcggtagatctctctacactctctttcagattatgacgttggaaagttggagtatggggatcgttcgacctgtaatggagagcttctcctatgcttgggcgtttttcatcccatttatccttattgctactttcaccatgcttaatctttttattgcaataattgttaatgcgatgcaaatggtctccgaagcggaccggtgtaatgctgcacagacccttgaacatcagagcgagcgcatagagggagagctccatgcagagatgggtaggctccgagtggagattcaggcgttgagagcaatgctttccatcacgcctgcgccggggcagactaaaccgtcatga

SEQ ID NO: 52 - DNA, 843 bp, synthetic construct
  misc_feature 1..843: note = Synthetic construct
  source 1..843: mol_type = other DNA
atgcaggaagctactctgccatctggtcagaacgtgatagaacggttgcgccggttggttgaatctaggcgctttacaggctttattacagccgtaatactgttcaacgcggtaactctgggacttgagacatggagttatgcaatggaagtggccgggggcctccttgttgccattgacagaatcgtattggctattttcgttttcgagatgatagcgaaactcttggtgtaccgccaggcgttctttcgcagcggttggaatatatttgaccttacaattgtgggcatcgcgcttgttcctgcggctggacccctcacagtgcttcgcgcgttgcggattctccgcgtgctgaggctcctgtcagtagttccgcaaatgaggtctgtggttgccgccctgattggcgccattccaggtatgggaagtatcgcagcggtcatgtccctcatattttatgttggatcagtacttgcaaccaaactgttcggggcggcgtttcctgactggtttgggtctattggggcgagtgcatatagtttgtttcagatcatgacgttggagtcatggagcatgggtatagtacgcccggtgatggaagtgtatccatgggcgtggctcttttttgttccgttcatcttgattacgacgttcgctgtgctgaacttggtggtggctgtaatagttaacagcatgcagacgcttcatgaggcggagcagaaggaagaaagagaagcagagaggcagatcgttcacgaagagacggccgctctcacgggggaggttagggcgatgaggcaggagctttcagaaataaaggcccttttgggggcaaaggcttga

SEQ ID NO: 53 - DNA, 819 bp, synthetic construct
  misc_feature 1..819: note = Synthetic construct
  source 1..819: mol_type = other DNA
atgcgcgaaaagatgctggtgcttaccaagtccagagagtgggagtctttcatccttattgtcataataattaacgcaatcacgctcggatttgaaacatctgaaactatcatgcaatccttcgcgggtccggccctccgattgtttgaccgggcggtcttggttatctttgtcgttgagatagctattcgcatttatgcgcatcgccttaggtttttccgggacccatggagtatcttcgatttcaccatcgtggtaatttcacttcttccagcgtccgggccacttcaagtcctccgggcactgcgaatactgcgagctcttaggctgctcagtatgattccttctctgaggcgggttatcggcggtcttattgctgctttgccgggaatggggtcaataattgttctcatggcgctggtcttttacatattcgcagtaatagccaccaaactgtatggggaggctttccccgagtggtttggtagtcttggcgcgacaatttatagtctgtttcagattatgactttggagtcttggtctatgggaatagttcgaccggtgatggaggtctacccgaacgcttggttgttttttgttcccttcatcctcagtacggcgttcaccgttcttaacttgtttattggcattatagtcagcgcgatgcagaaagagcatgaagaggaactgagagaagaggatcggcaggctagagaaccagagatgcaagaactgctccatgaggttagggcccttaggtcagaagtagctgctcttaggcaggatcaggccccacgaccggcacccacaacggcttga

SEQ ID NO: 54 - DNA, 840 bp, synthetic construct
  misc_feature 1..840: note = Synthetic construct
  source 1..840: mol_type = other DNA
atgacggaaattacgggtaccgtcgaaagaagtctgcaacagcaggttgcaacgtggcttcaaaaaaactgggttcaacgctctctcctgagcctcatacttataaacgcagtcattctcgggctggagacagcccctggtgttatggcagtagcaggagccccccttatgctccttgacaagttgatccttgccgttttcgtactcgaaatcgccctccgcatctttgcttacaggggcgcgtttttcaaagacgcttggtctctttttgatttcactgtggtggccatcgccctcgtcccggcctccggtccatttgccgttctgcgggctctcagagttttgagggtcctccgcgttctcacgttcgttccatcaatgaagaaaatagttggcgcgcttgtccaatcactcaacggaatgctctctatcgctatggtccttgggcttgtatattatgttagtgccgtaatggccacgaagctgtttggcgaggcttttcccgagtggtttggcaacatcggaagaacactttacacgctctttcaaataatgacgttggagagttggagtatgggcatttccaggcctgtcatggagcagttcccatatgcctgggcattcttcgtaccgtttatcctgatcgcaacattcaccatgttgaacctcttcatagcagtaatagtaaacgcagtacaatccatgcacgatgaagagcacaaggaggaaatagacgcgaaacagcagttgcaacacgaccttgtttcacaaatgcaacaacttcaagctgagctcgcggccctgagggcgcaattgccgccaaacaacaaagttgattga

SEQ ID NO: 55 - DNA, 834 bp, synthetic construct
  misc_feature 1..834: note = Synthetic construct
  source 1..834: mol_type = other DNA
atgaactctgacactatagtaactgcggtgccggtgcgccaacggttgcaacaatttatagaacatggtaccgttcagagaatgctgctcgcgctgatactcctgaatgcattcacactcggactggaaacctccaatgccgtaatgtctcttgcaggcactgcaatccatctccttgacaaagctattctcgctatattcgtccttgaaatattggtcagattgtatgtccatcgacttgctttcttcaaagatgcctggtccgttttcgacttcgtcgtggtaggtatagcccttctccctgcgagcggtccattctccgtgcttagagcactgcgggtacttcgggtcttgcgagtgcttacctttgttcctagtatgaagaagattgttggagcactcatgcagagcctgaacggaatgttgtccattgctatggttttgggactcgtttactacgttgcatccgtgatggttactaagctgtttggagctgctttccccgagtggttcggctcattgggagcctcactgtacaccctctttcaaataatgactctggagagttggagcatggggattgcccggccggtaatggagcaattcccttacgcctggctctttttcgtccctttcatcctcattgcaacattcacaatgctcaacctgtttatcgcggtcatcgtcaatgctgtacaatccatgcatgacgcagaacacaagacagaacaagacgccgagaaggcgacacagttgcaactcttgcaacagatgcaacagctcaagcagcagctgtctgaggtgcagcaacagcttagggaccggagtaactga

SEQ ID NO: 56 - DNA, 873 bp, synthetic construct
  misc_feature 1..873: note = Synthetic construct
  source 1..873: mol_type = other DNA
atgtttcacactcctggtgtaaaccccggactccgggaacgggcgggtagatggatagaatcaggacccgttcaacgagtaattatcgctctgattttgatcaatgctgccatactcggattggagacagatcccgacattatggctaggattggggattggctcattggggcggatagggtgattctgggtgtgttcgtagttgaaattttgatcaaattgtatgcaaaaggactccgctttttcagaaatccgtggaatgtatttgactttctcgtggtgggaattgcgttgatacccgccagtggcccgtttgccgttctgcgaatattgaggctcctgcgccttgtgtctatgattcctaagttgaggtttgtcgtggaagctctcttgagggcaatccctgggatcgccagcatatttgggctgctgataatccttttttacgttttcgcagttatcgcaaccggcttgtttgccaaagatcatcctgagtggtttggatcaatcgggcgatccatgtatactctgttccaagttatgacactcgaatcctggtcaatgggaattgctcggcctgtgatggagacgcatccctacgcatgggtgttcttcgtgcctttcattcttgtggcgaccttcacaatactcaatctgtttattgccataattgttaatactatgcagacacttgctgaggagcagcagaagttcgaagagaaaacaataacaacagttgtccacgcagagtcagcgcagctgcatcaggatcttacgagagttgagagcgagaaccaacaacttcaccaggatctgagggccctgagggaggagatccgagctttgcgcgaggaacttagaagacctggttga

SEQ ID NO: 57 - DNA, 855 bp, synthetic construct
  misc_feature 1..855: note = Synthetic construct
  source 1..855: mol_type = other DNA
atgaatgctcaacttcttggggacaccaccggcttccgagctaaagcacatcagttcattgagaacccattcatacaaaacggtattttggtcctgatcgtgattaatgccataacattggggctcgaaactgtcccggccgcgatgcagagattctcaaacataatacatacccttgatctcgtaatattgagtgtgttcgttcttgaactccttatacggctttatgtttatcgagagaaatactttaacgacccctggagagcttttgattttgtagtcgtgtcaattgcccttgtgcctgcaacgggccaactggctgtgctcagggcgctgagggttctccgagtgcttagaataataacaattgtgccctctatgaggcgggtggtgggggccttgttgagcgcaatacccggcttgacctcaatcgcgcttgttctcggcctgatatattatgtgttcgccgtgatagcgacaaacctgtttgctgccgagttcccagagtggttcggacatcttggccgctctttctacacactttttcagattatgacacttgaatcctggagtatgggtatagcgcggcctgttatggaaacttttccttatgcatgggccttttttataccgtttatcttggtcgcaactttcacgatgctcaacctctttattgcaattatagtgaatgccatgcagacgtttaccgagcaagaaaaacagggtaccgtcgaagccgtcaacgaggcccgcgaccatatagaggaagatatgcacacggagatgcgagccttgcgccgggagatcgctgagctgaagagcatgattcgaggtcaatacaggcaggacccgtga

SEQ ID NO: 58 - DNA, 849 bp, synthetic construct
  misc_feature 1..849: note = Synthetic construct
  source 1..849: mol_type = other DNA
atggctaatttgacagatagtgcgggaaatcccgggcatcgcgcgtggttgagagaatgggttgagtctgccccctttcgctataccgtccttgttataatattcatcaacgccatagtgctgggccttgaaaccgaggcttcagtcatagccgaagtcggggatatgcttcatttgattgacaagataatattgtggatattcgttgttgagttgatcctcaggatgtacgcgcatggtccacgattcttcctggacccttggggtgtattcgattttattatagtagccatagccttgtttcccgcctctgaagaatttagtgtcctccgagccttgcgcatactccgagcgttgcggctgatttccggtgtcccacgaatgcgcagggtcgtcgaagctctgctccgagcggtcccagggattggttctgtggctgctcttttgctcctggtcttctatgtcttcagtgtgatcgccactaaactgtttggcactgctttcccacagtggttcggaaccataggggaaagtatgtactccctgttccagattatgaccctggaaagctggtcaatgggaatcgtaaggccggtcatggaggaataccccgaagcctgggccttttttgttccgttcatcataatttccagttttaccgttctgaatttgtttatagctatcatcgtggattcaatgcagaccctccatgccgacgaggaggaacgcaccgtcgaaaggattgaaactattgtggacgaggatacgcagcttgtgagtgatgaaatcgcaaggcttcgggccgagattcgcgacttgaggagtgaactcaatggcaggaaaagttga

SEQ ID NO: 59 - protein, 17 aa, synthetic construct
  REGION 1..17: note = Synthetic construct
RSFVKKDGHCNVQFINV

SEQ ID NO: 60 - protein, 6 aa, synthetic construct
  REGION 1..6: note = Synthetic construct
DLRRSL

SEQ ID NO: 61 - protein, 6 aa, synthetic construct
  REGION 1..6: note = Synthetic construct
DLRRSL

SEQ ID NO: 62 - protein, 7 aa, synthetic construct
  REGION 1..7: note = Synthetic construct
FCYENEV

SEQ ID NO: 63 - protein, 20 aa, synthetic construct
  REGION 1..20: note = Synthetic construct
KSRITSEGEYIPLDQIDINV

SEQ ID NO: 64-67 - skipped (4 entries)

SEQ ID NO: 68 - protein, 9 aa, synthetic construct
  REGION 1..9: note = Synthetic construct
VPIAVAESD

SEQ ID NO: 69 - protein, 4 aa, synthetic construct
  REGION 1..4: note = Synthetic construct
YSVL

SEQ ID NO: 70 - skipped

SEQ ID NO: 71 - protein, 10 aa, synthetic construct
  REGION 1..10: note = Synthetic construct
MLCCMRRTKQ

SEQ ID NO: 72 - protein, 14 aa, synthetic construct
  REGION 1..14: note = Synthetic construct
KDNTTLQEFATLAN

SEQ ID NO: 73 - protein, 11 aa, synthetic construct
  REGION 1..11: note = Synthetic construct
PSSGHSRYALI

SEQ ID NO: 74-75 - skipped (2 entries)

SEQ ID NO: 76 - protein, 5 aa, synthetic construct
  REGION 1..5: note = Synthetic construct
  REGION 1..5: note = Gly-Gly-Gly-Gly-Ser - Gly-Gly-Gly-Gly-Ser at positions 1 to 5 may repeat from 1 to 10 times
GGGGS

SEQ ID NO: 77 - protein, 5 aa, synthetic construct
  REGION 1..5: note = Synthetic construct
  REGION 1..5: note = Glu-Ala-Ala-Ala-Lys - Glu-Ala-Ala-Ala-Lys at positions 1 to 5 may repeat from 1 to 10 times
EAAAK

SEQ ID NO: 78 - skipped

SEQ ID NO: 79 - protein, 427 aa, Homo sapiens
MGSVRTNRYSIVSSEEDGMKLATMAVANGFGNGKSKVHTRQQCRSRFVKKDGHCNVQFINVGEKGQRYLADIFTTCVDIRWRWMLVIFCLAFVLSWLFFGCVFWLIALLHGDLDASKEGKACVSEVNSFTAAFLFSIETQTTIGYGFRCVTDECPIAVFMVVFQSIVGCIIDAFIIGAVMAKMAKPKKRNETLVFSHNAVIAMRDGKLCLMWRVGNLRKSHLVEAHVRAQLLKSRITSEGEYIPLDQIDINVGFDSGIDRIFLVSPITIVHEIDEDSPLYDLSKQDIDNADFEIVVILEGMVEATAMTTQCRSSYLANEILWGHRYEPVLFEEKHYYKVDYSRFHKTYEVPNTPLCSARDLAEKKYILSNANSFCYENEVALTSKEEDDSENGVPESTSTDTPPDIDLHNQASVPLEPRPLRRESEI

SEQ ID NO: 80 - protein, 381 aa, Homo sapiens
MGDWSALGKLLDKVQAYSTAGGKVWLSVLFIFRILLLGTAVESAWGDEQSAFRCNTQQPGCENVCYDKSFPISHVRFWVLQIIFVSVPTLLYLAHVFYVMRKEEKLNKKEEELKVAQTDGVNVDMHLKQIEIKKFKYGIEEHGKVKMRGGLLRTYIISILFKSIFEVAFLLIQWYIYGFSLSAVYTCKRDPCPHQVDCFLSRPTEKTIFIIFMLWSLVSLALNIIELFYVFFKGVKDRVKGKSDPYHATSGALSPAKDCGSQKYAYFNGCSSPTAPLSPMSPPGYKLVTGDRNNSSCRNYNKQASEQNWANYSAEQNRMGQAGSTISNSHAQPFDFPDDNQNSKKLAAGHELQPLAIVDQRPSSRASSRASSRPRPDDLEI